European Patent Specification EP 3 967 679 B1, published February 19, 2025. Title: Novel inhibitors of meprin alpha and beta. Applicant: Vivoryon Therapeutics AG. The sequence listing filed with the application follows.

SEQUENCE LISTING (4 sequences)

SEQ ID NO: 1 - protein, 8 aa, Artificial Sequence
  Substrate
  Site (7)..(7): Xaa corresponds to Lys modified with Dnp (2,4-dinitrophenyl)
YVAEAPXG

SEQ ID NO: 2 - protein, 8 aa, Artificial Sequence
  Substrate
  Site (7)..(7): Xaa corresponds to Lys modified with Dnp (2,4-dinitrophenyl)
YVADAPXG

SEQ ID NO: 3 - protein, 7 aa, Artificial Sequence
  Substrate
  Site (5)..(5): Xaa corresponds to DprDnp, i.e. Dpr (2,3-diaminopropionic acid) modified with Dnp (2,4-dinitrophenyl)
PLGLXAR

SEQ ID NO: 4 - protein, 11 aa, Artificial Sequence
  Substrate
  Site (11)..(11): Xaa corresponds to DprDnp, i.e. Dpr (2,3-diaminopropionic acid) modified with Dnp (2,4-dinitrophenyl)
LANAVRSSSRX